European Patent Application EP 4 459 281 A1, published November 6, 2024. Title: Detection method and Detection reagent. Applicant: SEKISUI MEDICAL CO., LTD. The sequence listing filed with the application follows.

SEQUENCE LISTING (37 sequences)

SEQ ID NO: 1 - protein, 9 aa, synthetic construct
  REGION 1..9: note = Heavy chain CDR1
GFSLSIYGM

SEQ ID NO: 2 - protein, 9 aa, synthetic construct
  REGION 1..9: note = Heavy chain CDR1
AFSLSIYGM

SEQ ID NO: 3 - protein, 9 aa, synthetic construct
  REGION 1..9: note = Heavy chain CDR1
GASLSIYGM

SEQ ID NO: 4 - protein, 9 aa, synthetic construct
  REGION 1..9: note = Heavy chain CDR1
GFALSIYGM

SEQ ID NO: 5 - protein, 9 aa, synthetic construct
  REGION 1..9: note = Heavy chain CDR1
GFSASIYGM

SEQ ID NO: 6 - protein, 9 aa, synthetic construct
  REGION 1..9: note = Heavy chain CDR1
GFSLAIYGM

SEQ ID NO: 7 - protein, 9 aa, synthetic construct
  REGION 1..9: note = Heavy chain CDR1
GFSLSAYGM

SEQ ID NO: 8 - protein, 9 aa, synthetic construct
  REGION 1..9: note = Heavy chain CDR1
GFSLSIAGM

SEQ ID NO: 9 - protein, 9 aa, synthetic construct
  REGION 1..9: note = Heavy chain CDR1
GFSLSIYAM

SEQ ID NO: 10 - protein, 9 aa, synthetic construct
  REGION 1..9: note = Heavy chain CDR1
GFSLSIYGA

SEQ ID NO: 11 - protein, 7 aa, synthetic construct
  REGION 1..7: note = Heavy chain CDR2
NVWWDDE

SEQ ID NO: 12 - protein, 7 aa, synthetic construct
  REGION 1..7: note = Heavy chain CDR2
AVWWDDE

SEQ ID NO: 13 - protein, 7 aa, synthetic construct
  REGION 1..7: note = Heavy chain CDR2
NAWWDDE

SEQ ID NO: 14 - protein, 7 aa, synthetic construct
  REGION 1..7: note = Heavy chain CDR2
NVAWDDE

SEQ ID NO: 15 - protein, 7 aa, synthetic construct
  REGION 1..7: note = Heavy chain CDR2
NVWADDE

SEQ ID NO: 16 - protein, 7 aa, synthetic construct
  REGION 1..7: note = Heavy chain CDR2
NVWWADE

SEQ ID NO: 17 - protein, 7 aa, synthetic construct
  REGION 1..7: note = Heavy chain CDR2
NVWWDAE

SEQ ID NO: 18 - protein, 7 aa, synthetic construct
  REGION 1..7: note = Heavy chain CDR2
NVWWDDA

SEQ ID NO: 19 - protein, 16 aa, synthetic construct
  REGION 1..16: note = Heavy chain CDR3
FCTRIGANYGNYPPFD

SEQ ID NO: 20 - protein, 16 aa, synthetic construct
  REGION 1..16: note = Heavy chain CDR3
ACTRIGANYGNYPPFD

SEQ ID NO: 21 - protein, 16 aa, synthetic construct
  REGION 1..16: note = Heavy chain CDR3
FATRIGANYGNYPPFD

SEQ ID NO: 22 - protein, 16 aa, synthetic construct
  REGION 1..16: note = Heavy chain CDR3
FCARIGANYGNYPPFD

SEQ ID NO: 23 - protein, 16 aa, synthetic construct
  REGION 1..16: note = Heavy chain CDR3
FCTAIGANYGNYPPFD

SEQ ID NO: 24 - protein, 16 aa, synthetic construct
  REGION 1..16: note = Heavy chain CDR3
FCTRAGANYGNYPPFD

SEQ ID NO: 25 - protein, 16 aa, synthetic construct
  REGION 1..16: note = Heavy chain CDR3
FCTRIAANYGNYPPFD

SEQ ID NO: 26 - protein, 16 aa, synthetic construct
  REGION 1..16: note = Heavy chain CDR3
FCTRIGAAYGNYPPFD

SEQ ID NO: 27 - protein, 16 aa, synthetic construct
  REGION 1..16: note = Heavy chain CDR3
FCTRIGANAGNYPPFD

SEQ ID NO: 28 - protein, 16 aa, synthetic construct
  REGION 1..16: note = Heavy chain CDR3
FCTRIGANYANYPPFD

SEQ ID NO: 29 - protein, 16 aa, synthetic construct
  REGION 1..16: note = Heavy chain CDR3
FCTRIGANYGAYPPFD

SEQ ID NO: 30 - protein, 16 aa, synthetic construct
  REGION 1..16: note = Heavy chain CDR3
FCTRIGANYGNAPPFD

SEQ ID NO: 31 - protein, 16 aa, synthetic construct
  REGION 1..16: note = Heavy chain CDR3
FCTRIGANYGNYAPFD

SEQ ID NO: 32 - protein, 16 aa, synthetic construct
  REGION 1..16: note = Heavy chain CDR3
FCTRIGANYGNYPAFD

SEQ ID NO: 33 - protein, 16 aa, synthetic construct
  REGION 1..16: note = Heavy chain CDR3
FCTRIGANYGNYPPAD

SEQ ID NO: 34 - protein, 12 aa, synthetic construct
  REGION 1..12: note = Light chain CDR1
QSLLNSSPRKNS

SEQ ID NO: 35 - protein, 8 aa, synthetic construct
  REGION 1..8: note = Light chain CDR3
KQSYNLYT

SEQ ID NO: 36 - protein, 8 aa, synthetic construct
  REGION 1..8: note = Light chain CDR3
AQSYNLYT

SEQ ID NO: 37 - protein, 8 aa, synthetic construct
  REGION 1..8: note = Light chain CDR3
AAAAAAAA